European Patent Specification EP 4 499 876 B1, published April 1, 2026. Title: METHOD FOR DETECTING MICROSATELLITE INSTABILITY IN CANCER PATIENT. Applicant: INSTITUT CURIE. Application WO. The sequence listing filed with the application follows.

SEQUENCE LISTING (20 sequences)

SEQ ID NO: 1 - DNA, 25 bp, synthetic construct
  misc_feature 1..25: note = M1 Forward primer
  source 1..25: mol_type = other DNA
agttctctgaatttgctctgaatta

SEQ ID NO: 2 - DNA, 24 bp, synthetic construct
  misc_feature 1..24: note = M1 Reverse primer
  source 1..24: mol_type = other DNA
acaagtacatccatagagttcaac

SEQ ID NO: 3 - DNA, 16 bp, synthetic construct
  misc_feature 1..16: note = M1 MS Probe
  source 1..16: mol_type = other DNA
tctctttttttttccc

SEQ ID NO: 4 - DNA, 18 bp, synthetic construct
  misc_feature 1..18: note = M1 REF probe
  source 1..18: mol_type = other DNA
ctggaactcttattatct

SEQ ID NO: 5 - DNA, 24 bp, synthetic construct
  misc_feature 1..24: note = M2 Forward primer
  source 1..24: mol_type = other DNA
tgcatttgtttgtgactgttttac

SEQ ID NO: 6 - DNA, 21 bp, synthetic construct
  misc_feature 1..21: note = M2 Reverse primer
  source 1..21: mol_type = other DNA
tctttccttgtcatcttgcgt

SEQ ID NO: 7 - DNA, 17 bp, synthetic construct
  misc_feature 1..17: note = M2 MS Probe
  source 1..17: mol_type = other DNA
agattgtttttttttcc

SEQ ID NO: 8 - DNA, 18 bp, synthetic construct
  misc_feature 1..18: note = M2 REF probe
  source 1..18: mol_type = other DNA
ctgctgatagacaaatcc

SEQ ID NO: 9 - DNA, 21 bp, synthetic construct
  misc_feature 1..21: note = M3 Forward primer
  source 1..21: mol_type = other DNA
ctcgctttaaggatatgtctg

SEQ ID NO: 10 - DNA, 22 bp, synthetic construct
  misc_feature 1..22: note = M3 Reverse primer
  source 1..22: mol_type = other DNA
gtggaacactgattagtaactg

SEQ ID NO: 11 - DNA, 16 bp, synthetic construct
  misc_feature 1..16: note = M3 MS Probe
  source 1..16: mol_type = other DNA
caggtttttttttgtc

SEQ ID NO: 12 - DNA, 16 bp, synthetic construct
  misc_feature 1..16: note = M3 REF probe
  source 1..16: mol_type = other DNA
ctatgatcgactaagt

SEQ ID NO: 13 - DNA, 20 bp, synthetic construct
  misc_feature 1..20: note = M4 Forward primer
  source 1..20: mol_type = other DNA
tgtggagcaaacagagggat

SEQ ID NO: 14 - DNA, 24 bp, synthetic construct
  misc_feature 1..24: note = M4 Reverse primer
  source 1..24: mol_type = other DNA
ttgctacttaccaaattgaagtgt

SEQ ID NO: 15 - DNA, 16 bp, synthetic construct
  misc_feature 1..16: note = M4 MS Probe
  source 1..16: mol_type = other DNA
ccctaaaaaaaaatgt

SEQ ID NO: 16 - DNA, 15 bp, synthetic construct
  misc_feature 1..15: note = M4 REF probe
  source 1..15: mol_type = other DNA
cttacttttcccact

SEQ ID NO: 17 - DNA, 40 bp, synthetic construct
  misc_feature 1..40: note = M1 sequence
  source 1..40: mol_type = other DNA
tttatttgatttttctctctttttttttcccccttgtatt

SEQ ID NO: 18 - DNA, 40 bp, synthetic construct
  misc_feature 1..40: note = M2 sequence
  source 1..40: mol_type = other DNA
atctcaagattgtttttttttccccttcagatacgcaaga

SEQ ID NO: 19 - DNA, 40 bp, synthetic construct
  misc_feature 1..40: note = M3 sequence
  source 1..40: mol_type = other DNA
acattttccaggtttttttttgtcattctatgatcgacta

SEQ ID NO: 20 - DNA, 40 bp, synthetic construct
  misc_feature 1..40: note = M4 sequence
  source 1..40: mol_type = other DNA
taaagttgccctaaaaaaaaatgtacagcttttcttactt